European Patent Application EP 4 656 248 A2, published December 3, 2025. Title: ANTI-C-MET ANTIBODY DRUG CONJUGATES. Applicant: AbbVie Manufacturing Management Unlimited Company. Application EP. The sequence listing filed with the application follows.

SEQUENCE LISTING (28 sequences)

SEQ ID NO: 1 - protein, 8 aa, synthetic construct
  REGION 1..8: note = Synthetic polypeptide
GYIFTAYT

SEQ ID NO: 2 - protein, 8 aa, synthetic construct
  REGION 1..8: note = Synthetic polypeptide
IKPNNGLA

SEQ ID NO: 3 - protein, 11 aa, synthetic construct
  REGION 1..11: note = Synthetic polypeptide
ARSEITTEFDY

SEQ ID NO: 4 - protein, 10 aa, synthetic construct
  REGION 1..10: note = Synthetic polypeptide
ESVDSYANSF

SEQ ID NO: 5 - skipped

SEQ ID NO: 6 - protein, 9 aa, synthetic construct
  REGION 1..9: note = Synthetic polypeptide
QQSKEDPLT

SEQ ID NO: 7 - protein, 118 aa, synthetic construct
  REGION 1..118: note = Synthetic polypeptide
QVQLVQSGAEVKKPGASVKVSCKASGYIFTAYTMHWVRQAPGQGLEWMGWIKPNNGLANYAQKFQGRVTMTRDTSISTAYMELSRLRSDDTAVYYCARSEITTEFDYWGQGTLVTVSS

SEQ ID NO: 8 - protein, 111 aa, synthetic construct
  REGION 1..111: note = Synthetic polypeptide
DIVMTQSPDSLAVSLGERATINCKSSESVDSYANSFLHWYQQKPGQPPKLLIYRASTRESGVPDRFSGSGSGTDFTLTISSLQAEDVAVYYCQQSKEDPLTFGGGTKVEIK

SEQ ID NO: 9 - protein, 445 aa, synthetic construct
  REGION 1..445: note = Synthetic polypeptide
QVQLVQSGAEVKKPGASVKVSCKASGYIFTAYTMHWVRQAPGQGLEWMGWIKPNNGLANYAQKFQGRVTMTRDTSISTAYMELSRLRSDDTAVYYCARSEITTEFDYWGQGTLVTVSSASTKGPSVFPLAPSSKSTSGGTAALGCLVKDYFPEPVTVSWNSGALTSGVHTFPAVLQSSGLYSLSSVVTVPSSSLGTQTYICNVNHKPSNTKVDKRVEPKSCDCHCPPCPAPELLGGPSVFLFPPKPKDTLMISRTPEVTCVVVDVSHEDPEVKFNWYVDGVEVHNAKTKPREEQYNSTYRVVSVLTVLHQDWLNGKEYKCKVSNKALPAPIEKTISKAKGQPREPQVYTLPPSREEMTKNQVSLTCLVKGFYPSDIAVEWESNGQPENNYKTTPPVLDSDGSFFLYSKLTVDKSRWQQGNVFSCSVMHEALHNHYTQKSLSLSPG

SEQ ID NO: 10 - protein, 218 aa, synthetic construct
  REGION 1..218: note = Synthetic polypeptide
DIVMTQSPDSLAVSLGERATINCKSSESVDSYANSFLHWYQQKPGQPPKLLIYRASTRESGVPDRFSGSGSGTDFTLTISSLQAEDVAVYYCQQSKEDPLTFGGGTKVEIKRTVAAPSVFIFPPSDEQLKSGTASVVCLLNNFYPREAKVQWKVDNALQSGNSQESVTEQDSKDSTYSLSSTLTLSKADYEKHKVYACEVTHQGLSSPVTKSFNRGEC

SEQ ID NO: 11 - protein, 460 aa, synthetic construct
  REGION 1..460: note = Synthetic polypeptide
EEQVLESGGGLVKPGGSLRLSCAASGFTFSPYSVFWVRQAPGKGLEWVSSINSDSTYKYYADSVKGRFTISRDNAENSIFLQMNSLRAEDTAVYYCARDRSYYAFSSGSLSDYYYGLDVWGQGTTVIVSSASTKGPSVFPLAPSSKSTSGGTAALGCLVKDYFPEPVTVSWNSGALTSGVHTFPAVLQSSGLYSLSSVVTVPSSSLGTQTYICNVNHKPSNTKVDKKVEPKSCDKTHTCPPCPAPEAAGGPSVFLFPPKPKDTLMISRTPEVTCVVVDVSHEDPEVKFNWYVDGVEVHNAKTKPREEQYNSTYRVVSVLTVLHQDWLNGKEYKCKVSNKALPAPIEKTISKAKGQPREPQVYTLPPSRDELTKNQVSLTCLVKGFYPSDIAVEWESNGQPENNYKTTPPVLDSDGSFFLYSKLTVDKSRWQQGNVFSCSVMHEALHNHYTQKSLSLSPGK

SEQ ID NO: 12 - protein, 219 aa, synthetic construct
  REGION 1..219: note = Synthetic polypeptide
DIVMTQSPLSLSVTPGEPASISCRSSQSLLHTNGYNYLDWYVQKPGQSPQLLIYLASNRASGVPDRFSGSGSGTDFTLKISRVETEDVGVYYCMQALQIPRTFGQGTKVEIKRTVAAPSVFIFPPSDEQLKSGTASVVCLLNNFYPREAKVQWKVDNALQSGNSQESVTEQDSKDSTYSLSSTLTLSKADYEKHKVYACEVTHQGLSSPVTKSFNRGEA

SEQ ID NO: 13 - protein, 118 aa, synthetic construct
  REGION 1..118: note = Synthetic polypeptide
EVQLQQSGPELVKPGASVKISCKTSGYIFTAYTMHWVRQSLGESLDWIGGIKPNNGLANYNQKFKGKATLTVDKSSSTAYMDLRSLTSEDSAVYYCARSEITTEFDYWGQGTALTVSS

SEQ ID NO: 14 - protein, 111 aa, synthetic construct
  REGION 1..111: note = Synthetic polypeptide
DIVLTQSPASLAVSLGQRATISCRASESVDSYANSFMHWYQQKPGQPPKLLIYRASNLESGIPARFSGSGSRTDFTLTINPVEADDVATYYCQQSKEDPLTFGSGTKLEMK

SEQ ID NO: 15 - protein, 8 aa, synthetic construct
  REGION 1..8: note = Synthetic polypeptide
GYIFTAYT

SEQ ID NO: 16 - protein, 8 aa, synthetic construct
  REGION 1..8: note = Synthetic polypeptide
IKPNNGLA

SEQ ID NO: 17 - protein, 11 aa, synthetic construct
  REGION 1..11: note = Synthetic polypeptide
ARSEITTEFDY

SEQ ID NO: 18 - protein, 10 aa, synthetic construct
  REGION 1..10: note = Synthetic polypeptide
ESVDSYANSF

SEQ ID NO: 19 - skipped

SEQ ID NO: 20 - protein, 9 aa, synthetic construct
  REGION 1..9: note = Synthetic polypeptide
QQSKEDPLT

SEQ ID NO: 21 - DNA, 1395 bp, synthetic construct
  misc_feature 1..1395: note = Synthetic polynucleotide
  source 1..1395: mol_type = other DNA
atgggatggtcttggatctttctgctgtttctgtctggtactgctggtgtgctgagccaggtccagctggtgcaatccggcgcagaggtgaagaagccaggcgcttccgtgaaggtgagctgtaaggcctctggctacatcttcacagcatacaccatgcactgggtgaggcaagctcctgggcagggactggagtggatgggatggattaaacccaacaatgggctggccaactacgcccagaaattccagggtagggtcactatgacaagggataccagcatcagcaccgcatatatggagctgagcaggctgaggtctgacgacactgctgtctattattgcgccaggagcgaaattacaacagaattcgattactgggggcagggcaccctggtgaccgtgtcctctgccagcaccaagggcccaagcgtgttccccctggcccccagcagcaagagcaccagcggcggcacagccgccctgggctgcctggtgaaggactacttccccgagcccgtgaccgtgtcctggaacagcggagccctcacttctggagttcataccttcccagcagtattgcagagcagtggcctgtattcactgtcttccgtcgtaacagttccatcctccagcctcgggacacagacttacatttgtaacgtgaatcacaagcctagcaacaccaaggtcgacaagagagttgaaccaaagagttgtgattgccactgtcctccctgcccagctcctgagctgcttggcggtcccagtgtcttcttgtttccccctaaacccaaagacaccctgatgatctcaaggactcccgaggtgacatgcgtggtggtggatgtgtctcatgaggacccagaggtgaagttcaactggtacgtggacggcgtggaggtgcacaacgccaagaccaagcccagagaggagcagtacaacagcacctacagggtggtgtccgtgctgaccgtgctgcaccaggactggctgaacggcaaggagtacaagtgtaaggtgtccaacaaggccctgccagccccaatcgaaaagaccatcagcaaggccaagggccagccaagagagccccaggtgtacaccctgccacccagcagggaggagatgaccaagaaccaggtgtccctgacctgtctggtgaagggcttctacccaagcgacatcgccgtggagtgggagagcaacggccagcccgagaacaactacaagaccacccccccagtgctggacagcgacggcagcttcttcctgtacagcaagctgaccgtggacaagagcagatggcagcagggcaacgtgttcagctgctccgtgatgcacgaggccctgcacaaccactacacccagaagagcctgagcctgtccccaggctga

SEQ ID NO: 22 - DNA, 24 bp, synthetic construct
  misc_feature 1..24: note = Synthetic polynucleotide
  source 1..24: mol_type = other DNA
ggctacatcttcacagcatacacc

SEQ ID NO: 23 - DNA, 24 bp, synthetic construct
  misc_feature 1..24: note = Synthetic polynucleotide
  source 1..24: mol_type = other DNA
attaaacccaacaatgggctggcc

SEQ ID NO: 24 - DNA, 33 bp, synthetic construct
  misc_feature 1..33: note = Synthetic polynucleotide
  source 1..33: mol_type = other DNA
gccaggagcgaaattacaacagaattcgattac

SEQ ID NO: 25 - DNA, 717 bp, synthetic construct
  misc_feature 1..717: note = Synthetic polynucleotide
  source 1..717: mol_type = other DNA
atggaaactgatacactgctgctgtgggtcctgctgctgtgggtccctggaagcacaggggacattgtgatgacccagtctcccgatagcctggccgtgtccctgggcgagagggctaccatcaactgtaaaagctccgaatctgtggactcttacgcaaacagctttctgcactggtatcagcaaaagccaggccaacctccaaagctgctgatttacagggcttctaccagggagagcggcgtgcccgataggttcagcggatctggcagcggcaccgactttacactgaccatctccagcctgcaggccgaagatgtggcagtctattactgccagcagtccaaggaggaccccctgactttcgggggtggtactaaagtggagatcaagcgtacggtggccgctcccagcgtgttcatcttccccccaagcgacgagcagctgaagagcggcaccgccagcgtggtgtgtctgctgaacaacttctaccccagggaggccaaggtgcagtggaaggtggacaacgccctgcagagcggcaacagccaggagagcgtcaccgagcaggacagcaaggactccacctacagcctgagcagcaccctgaccctgagcaaggccgactacgagaagcacaaggtgtacgcctgtgaggtgacccaccagggcctgtccagccccgtgaccaagagcttcaacaggggcgagtgctga

SEQ ID NO: 26 - DNA, 30 bp, synthetic construct
  misc_feature 1..30: note = Synthetic polynucleotide
  source 1..30: mol_type = other DNA
gaatctgtggactcttacgcaaacagcttt

SEQ ID NO: 27 - skipped

SEQ ID NO: 28 - DNA, 27 bp, synthetic construct
  misc_feature 1..27: note = Synthetic polynucleotide
  source 1..27: mol_type = other DNA
cagcagtccaaggaggaccccctgact